European Patent Specification EP 3 953 367 B1, published February 11, 2026. Title: VERSATILE PEPTIDE AND PROTEIN MACROCYCLIZATION AND MULTIMERIZATION WITH DIELS-ALDER CYCLOADDITIONS. Applicant: The University of Chicago. The sequence listing filed with the application follows.

SEQUENCE LISTING (12 sequences)

SEQ ID NO: 1 - protein, 5 aa, Artificial Sequence
  Synthetic Sequence
  misc_feature (1)..(1): Xaa is C(hex)
  misc_feature (5)..(5): Xaa is K(mal)
XRGDX

SEQ ID NO: 2 - protein, 5 aa, Artificial Sequence
  Synthetic Sequence
  misc_feature (1)..(1): Xaa is C(hex)
  misc_feature (5)..(5): Xaa is K(mal)
XVGDX

SEQ ID NO: 3 - protein, 6 aa, Artificial Sequence
  Synthetic Sequence
  misc_feature (1)..(1): Xaa is C(hex)
  misc_feature (6)..(6): Xaa is K(mal)
XAPVYX

SEQ ID NO: 4 - protein, 8 aa, Artificial Sequence
  Synthetic Sequence
  misc_feature (1)..(1): Xaa is C(hex)
  misc_feature (8)..(8): Xaa is K(mal)
XAVPAVYX

SEQ ID NO: 5 - protein, 5 aa, Artificial Sequence
  Synthetic Sequence
  misc_feature (2)..(3): Xaa can be any naturally occurring amino acid
LXXLL

SEQ ID NO: 6 - protein, 21 aa, Artificial Sequence
  Synthetic Sequence
SCFGGRMDRIGAQSGLGCNSF

SEQ ID NO: 7 - protein, 21 aa, Artificial Sequence
  Synthetic Sequence
  misc_feature (7)..(7): Xaa is AA with dienophile
  misc_feature (14)..(14): Xaa is AA with diene
SCFGGRXDRIGAQXGLGCNSF

SEQ ID NO: 8 - protein, 21 aa, Artificial Sequence
  Synthetic Sequence
  misc_feature (7)..(7): Xaa is C(hex)
  misc_feature (14)..(14): Xaa is K(mal)
SCFGGRXDRIGAQXGLGCNSF

SEQ ID NO: 9 - protein, 24 aa, Artificial Sequence
  Synthetic Sequence
  misc_feature (22)..(22): Xaa is beta-alanine
  misc_feature (23)..(23): Xaa is K(mmt)
KRAHHNALERKRRDHIKDSFHXXW

SEQ ID NO: 10 - protein, 21 aa, Artificial Sequence
  Synthetic Sequence
  misc_feature (3)..(3): Xaa is S5
  misc_feature (7)..(7): Xaa is S5
  misc_feature (20)..(20): Xaa is beta-alanine
  misc_feature (21)..(21): Xaa is K(mmt)
KRXHHNXLERKRRDHIKDSXX

SEQ ID NO: 11 - protein, 24 aa, Artificial Sequence
  Synthetic Sequence
  misc_feature (22)..(22): Xaa is beta-alanine
  misc_feature (22)..(23): Xaa is K(cpd)
KRAHHNALERKRRDHIKDSFHXXW

SEQ ID NO: 12 - protein, 21 aa, Artificial Sequence
  Synthetic Sequence
  misc_feature (3)..(3): Xaa is S5
  misc_feature (7)..(7): Xaa is S5
  misc_feature (20)..(20): Xaa is beta-alanine
  misc_feature (21)..(21): Xaa is K(cpd)
KRXHHNXLERKRRDHIKDSXX